European Patent Application EP 4 707 810 A1, published March 11, 2026. Title: USE OF GLUT1 AS A MARKER FOR HEMATOLOGIC DISORDERS. Applicant: METAFORA BIOSYSTEMS. The sequence listing filed with the application follows.

SEQUENCE LISTING (71 sequences)

SEQ ID NO: 1 - DNA, 18 bp, synthetic construct
  source 1..18: mol_type = other DNA
tctcccagcgtgcgccat

SEQ ID NO: 2 - protein, 189 aa, synthetic construct
MALPYHIFLFTVVSPSFTLTAPPPCRCMTSSSPYQEFLWRMQRPGNIDAPSYRSLCKGTPTFTAHTHMPRNCYHSATLCMHANTHYWTGKMINPSCPGGLGVTVCWTYFTQTGMSDGGGVQDQAREKHVKEVISQLTRVHGTSSPYKGLDLSKLHETLRTHTRLVSLFNTTLTGLHEVSAQNPTNCWIC

SEQ ID NO: 3 - protein, 189 aa, synthetic construct
MALPYHIFLFTVLLPSFTLTAPPPCRCMTSSSPYQEFLWRMQRPGNIDAPSYRSLCKGTPTFTAHTHMPRNCYHSATLCMHANTHYWTGKMINPSCPGGLGVTVCWTYFTQTGMSDGGGVQDQAREKHVKEVISQLTRVHGTSSPYKGLDLSKLHETLRTHTRLVSLFNTTLTGLHEVSAQNPTNCWIC

SEQ ID NO: 4 - protein, 121 aa, synthetic construct
MALPYHIFLFTVLLPSFTLTAPPPCRCMTSSSPYQEFLWRMQRPGNIDAPSYRSLSKGTPTFTAHTHMPRNCYHSATLCMHANTHYWTGKMINPSCPGGLGVTVCWTYFTQTGMSDGGGVQ

SEQ ID NO: 5 - protein, 181 aa, synthetic construct
MALPYHIFLFTVLLPSFTLTAPPPCRCMTSSSPYQEFLWRMQRPGNIDAPSYRSLSKGTPTFTAHTHMPRNCYHSATLCMHANTHYWTGKMINPSCPGGLGVTVCWTYFTQTGMSDGGGVQDQAREKHVKEVISQLTRVHGTSSPYKGLDLSKLHETLRTHTRLVSLFNTTLTGLHEVSAQ

SEQ ID NO: 6 - protein, 239 aa, synthetic construct
MKLPTGMVILCSLIIVRAGFDDPRKAIALVQKQHGKPCECSGGQVSEAPPNSIQQVTCPGKTAYLMTNQKWKCRVTPKISPSGGELQNCPCNTFQDSMHSSCYTEYRQCRRINKTYYTATLLKIRSGSLNEVQILQNPNQLLQSPCRGSINQPVCWSATAPIHISDGGGPLDTKRVWTVQKRLEQIHKAMTPELQYHPLALPKVRDDLSLDARTFDILNTTFRLLQMSNFSLAQDCWLC

SEQ ID NO: 7 - protein, 222 aa, synthetic construct
MKLPTGMVILCSLIIVRAGFDDPRKAIALVQKQHGKPCECSGGQVSEAPPNSIQQVTCPGKTAYLMTNQKWKCRVTPKISPSGGELQNCPCNTFQDSMHSSCYTEYRQCRRINKTYYTATLLKIRSGSLNEVQILQNPNQLLQSPCRGSINQPVCWSATAPIHISDGGGPLDTKRVWTVQKRLEQIHKAMTPELQYHPLALPKVRDDLSLDARTFDILNTTF

SEQ ID NO: 8 - protein, 223 aa, synthetic construct
MKLPAGMVILCSLIIVRAGFDDPRKAIALVQKQHGKPCECSGGQVSEAPPNSIQQVTCPGKTAYLMTNQKWKCRVTPKNLTPSGGELQNCPCNTFQDSMHSSCYTEYRQCRANNKTYYTATLLKIRSGSLNEVQILQNPNQLLQSPCRGSINQPVCWSATAPIHISDGGGPLDTKRVWTVQKRLEQIHKAMHPELQYHPLALPKVRDDLSLDARTFDILNTTF

SEQ ID NO: 9 - protein, 331 aa, synthetic construct
MKPPAGMVFLWVLTSLGAGIGAKIVKEGNPHQVYTLTWQIYSQSGEVVWEVQGNHALNTWWPPLTPDFCQLAAGLDTWDIPARSPKNLQSYMGERIQQMTAHGCSSPTARCRLAQAEFYVCPRDNRDRATAHRCGGYEEYFCSAWGCETTGDAYWQPTSSWDLITITRGYTKPDPDGHTCYYKKGTEGYHHWISPLSLPLKITFTDSGKRALGWQTGYTWGLRWYLPGKDRGIVLKIKLKIDTITQTVGPNLVLADQKAPVQLAIPVQPPRAPTQTPGINPVNSTLSPSLGYPTPPLDRAQGDRLLNLVQGVYLTLNLTAPNQTQDCWLCL

SEQ ID NO: 10 - protein, 222 aa, synthetic construct; identical to SEQ ID NO: 7

SEQ ID NO: 11 - protein, 239 aa, synthetic construct
MGFTTKIIFLYNLVLVYAGFDDPRKAIELVQKRYGRPCDCSGGQVSEPPSDRVSQVTCSGKTAYLMPDQRWKCKSIPKDTSPSGPLQECPCNSYQSSVHSSCYTSYQQCRSGNKTYYTATLLKTQTGGTSDVQVLGSTNKLIQSPCNGIKGQSICWSTTAPIHVSDGGGPLDTTRIKSVQRKLEEIHKALYPELQYHPLAIPKVRDNLMVDAQTLNILNATYNLLLMSNTSLVDDCWLC

SEQ ID NO: 12 - protein, 258 aa, synthetic construct
MDCLTNLRSAEGKVDQASKILILLVAWWGFGTTAEGYPLQQLWELPCDCSGGYVSSIPTYYTYSLDCGGSTAYLTYGSGTGSWSWGGGFKQQWECVFKPKIIPSVQGQPGPCPSECLQIATQMHSTCYEKTQECTLLGKTYFTAILQKTKLGSYEDGPNKLIQASCTGTVGKPVCWDPVAPVYVSDGGGPTDMIREESVRERLEEIIRHSYPSVQYHPLALPRSRGVDLDPQTSDILEATHQVLNATNPQLAENCWLC

SEQ ID NO: 13 - protein, 567 aa, synthetic construct
MDCLTNLRSAEGKVDQASKILILLVAWWGFGTTAEGYPLQQLWELPCDCSGGYVSSIPTYYTYSLDCGGSTAYLTYGSGTGSWSWGGGFKQQWECVFKPKIIPSVQGQPGPCPSECLQIATQMHSTCYEKTQECTLLGKTYFTAILQKTKLGSYEDGPNKLIQASCTGTVGKPVCWDPVAPVYVSDGGGPTDMIREESVRERLEEIIRHSYPSVQYHPLALPRSRGVDLDPQTSDILEATHQVLNATNPKLAENCWLCMTLGTPIPAAIPTNGNVTLDGNCSLSLPFGCNPPGSIDVSCYAGEADNRTGIPVGYVHFTNCTSIQEVTNETSQMGNLTRLCPPPGHVFVCGNNMAYTALPNKWIGLCILASIVPDISIISGEEPIPLPSIEYTARRHKRAVQFIPLLVGLGISGATLAGGTGLGVSVHTYHKLSNQLIEDVQALSGTINDLQDQIDSLAEVVLQNRRGLDLLTAEQGGICLALQEKCCFYANKSGIVRDKIRKLQEDLIERKRALYDNPLWSGLNGFLPYLLPLLGPLFGLILFLTLGPCIMKTLTRIIHDKIQAVKS

SEQ ID NO: 14 - protein, 251 aa, synthetic construct
MNFNHHFTWSLVIISQIFQVQAGFGDPREALLEIQQKHGKPCDCAGGYVSSPPTNSLTTVSCSTYTAYSVTNSLKWQCVSTPTTASPTHIGSCPSQCNSQSYDSVHATCYNHYQQCTIGNKTYLTATMIRDKSPSSGDGNVPTILGNNQNLIIAGCPENKKGQVVCWNSQPSVHMSDGGGPQDKVREIIVNKKFEELHKSLFPELSYHPLALPEARGKEKIDAHTFDLLATVHSLLNVSSQRQLAEDCWLC

SEQ ID NO: 15 - protein, 250 aa, synthetic construct
MNFNYHFIWSLVILSQISQVQAGFGDPREALAEIQQKHGKPCDCAGGYVSSPPINSLTTVSCSTHTAYSVTNSLKWQCVSTPTTPSNTHIGSCPGECNTISYDSVHASCYNHYQQCNIGNKTYLTATITGDRTPAIGDGNVPTVLGTSHNLITAGCPNGKKGQVVCWNSRPSVHISDGGGPQDKARDIIVNKKFEELHRSLFPELSYHPLALPEARGKEKIDAHTLDLLATVHSLLNASQPSLAEDCWLC

SEQ ID NO: 16 - protein, 312 aa, synthetic construct
MGKFLATLILFFQFCPLILGDYSPSCCTLTIGVSSYHSKPCNPAQPVCSWTLDLLALSADQALQPPCPNLVSYSSYHATYSLYLFPHWIKKPNRNGGGYYSASYSDPCSLKCPYLGCQSWTCPYTGAVSSPYWKFQQDVNFTQEVSRLNINLHFSKCGFPFSLLVDAPGYDPIWFLNTEPSQLPPTAPPLLPHSNLDHILEPSIPWKSKLLTLVQLTLQSTNYTCIVCIDRASLSTWHVLYSPNVSVPSSSSTPLLYPSLALPAPHLTLPFNWTHCFDPQIQAIVSSPCHNSLILPPFSLSPVPTLGSRSRR

SEQ ID NO: 17 - protein, 292 aa, synthetic construct
DYSPSCCTLTIGVSSYHSKPCNPAQPVCSWTLDLLALSADQALQPPCPNLVSYSSYHATYSLYLFPHWIKKPNRNGGGYYSASYSDPCSLKCPYLGCQSWTCPYTGAVSSPYWKFQQDVNFTQEVSRLNINLHFSKCGFPFSLLVDAPGYDPIWFLNTEPSQLPPTAPPLLPHSNLDHILEPSIPWKSKLLTLVQLTLQSTNYTCIVCIDRASLSTWHVLYSPNVSVPSSSSTPLLYPSLALPAPHLTLPFNWTHCFDPQIQAIVSSPCHNSLILPPFSLSPVPTLGSRSRR

SEQ ID NO: 18 - protein, 228 aa, synthetic construct
MGKFLATLILFFQFCPLIFGDYSPSCCTLTIGVSSYHSKPCNPAQPVCSWTLDLLALSADQALQPPCPNLVSYSSYHATYSLYLFPHWTKKPNRNGGGYYSASYSDPCSLKCPYLGCQSWTCPYTGAVSSPYWKFQHDVNFTQEVSRLNINLHFSKCGFPFSLLVDAPGYDPIWFLNTEPSQLPPTAPPLLPHSNLDHILEPSIPWKSKLLTLVQLTLQSTNYTCIVC

SEQ ID NO: 19 - protein, 182 aa, synthetic construct
MGKFLATLILFFQFCPLIFGDYSPSCCTLTIGVSSYHSKPCNPAQPVCSWTLDLLALSADQALQPPCPNLVSYSSYHATYSLYLFPHWTKKPNRNGGGYYSASYSDPCSLKCPYLGCQSWTCPYTGAVSSPYWKFQHDVNFTQEVSRLNINLHFSKCGFPFSLLVDAPGYDPIWFLNTEPSQ

SEQ ID NO: 20 - protein, 51 aa, synthetic construct
IKKPNPNGGGYYLASYSDPCSLKCPYLGCQSWTCPYTGAVSSPYWKFQQDV

SEQ ID NO: 21 - protein, 51 aa, synthetic construct
VKKPNRNGGGYYLASYSDPCSLKCPYLGCQSWTCPYTGAVSSPYWKFQQDV

SEQ ID NO: 22 - protein, 51 aa, synthetic construct
IKKPNRNGGGYYLASYSDPCSLKCPYLGCQSWTCPYTGAVSSPYWKFQQDV

SEQ ID NO: 23 - protein, 51 aa, synthetic construct
IKKPNRNGGGYYLASYSDPCSLKCPYLGCQSWTCPYTGPVSSPYWKFQQDV

SEQ ID NO: 24 - protein, 57 aa, synthetic construct
IKKPNRNGGGYHSASYSDPCSLKCPYLGCQSWTCPYAGAVSSPYWKFQQDVNFTQEV

SEQ ID NO: 25 - protein, 208 aa, synthetic construct
DYSPSCCTLTIGVSSYHSKPCNPAQPVCSWTLDLLALSADQALQPPCPNLVSYSSYHATYSLYLFPHWTKKPNRNGGGYYSASYSDPCSLKCPYLGCQSWTCPYTGAVSSPYWKFQHDVNFTQEVSRLNINLHFSKCGFPFSLLVDAPGYDPIWFLNTEPSQLPPTAPPLLPHSNLDHILEPSIPWKSKLLTLVQLTLQSTNYTCIVC

SEQ ID NO: 26 - protein, 162 aa, synthetic construct
DYSPSCCTLTIGVSSYHSKPCNPAQPVCSWTLDLLALSADQALQPPCPNLVSYSSYHATYSLYLFPHWTKKPNRNGGGYYSASYSDPCSLKCPYLGCQSWTCPYTGAVSSPYWKFQHDVNFTQEVSRLNINLHFSKCGFPFSLLVDAPGYDPIWFLNTEPSQ

SEQ ID NO: 27 - protein, 308 aa, synthetic construct
MGNVFFLLLFSLTHFPPVQQSRCTLTVGISSYHSSPCSPTQPVCTWNLDLNSLTTDQRLHPPCPNLITYSGFHKTYSLYLFPHWIKKPNRQGLGYYSPSYNDPCSLQCPYLGCQSWTCPYTGPVSSPSWKFHSDVNFTQEVSQVSLRLHFSKCGSSMTLLVDAPGYDPLWFITSEPTQPPPTPPPLVHDSDLEHVLTPSTSWTTKMLKFIQLTLQSTNYSCMVCVDRSSLSSWHVLYTPNISIPQQTSSRTILFPSLALPAPPFQPFPWTHCYQPRLQAITTDDCNNSIILPPFSLAPVPPPATRRRR

SEQ ID NO: 28 - protein, 288 aa, synthetic construct
SRCTLTVGISSYHSSPCSPTQPVCTWNLDLNSLTTDQRLHPPCPNLITYSGFHKTYSLYLFPHWIKKPNRQGLGYYSPSYNDPCSLQCPYLGCQSWTCPYTGPVSSPSWKFHSDVNFTQEVSQVSLRLHFSKCGSSMTLLVDAPGYDPLWFITSEPTQPPPTPPPLVHDSDLEHVLTPSTSWTTKMLKFIQLTLQSTNYSCMVCVDRSSLSSWHVLYTPNISIPQQTSSRTILFPSLALPAPPFQPFPWTHCYQPRLQAITTDDCNNSIILPPFSLAPVPPPATRRRR

SEQ ID NO: 29 - protein, 224 aa, synthetic construct
MGNVFFLLLFSLTHFPLAQQSRCTLTVGISSYHSSPCSPTQPVCTWNLDLNSLTTDQRLHPPCPNLITYSGFHKTYSLYLFPHWIKKPNRQGLGYYSPSYNDPCSLQCPYLGCQSWTCPYTGPVSSPSWKFHSDVNFTQEVSQVSLRLHFSKCGSSMTLLVDAPGYDPLWFITSEPTQPPPTSPPLVHDSDLEHVLTPSTSWTTKILKFIQLTLQSTNYSCMVC

SEQ ID NO: 30 - protein, 178 aa, synthetic construct
MGNVFFLLLFSLTHFPLAQQSRCTLTVGISSYHSSPCSPTQPVCTWNLDLNSLTTDQRLHPPCPNLITYSGFHKTYSLYLFPHWIKKPNRQGLGYYSPSYNDPCSLQCPYLGCQSWTCPYTGPVSSPSWKFHSDVNFTQEVSQVSLRLHFSKCGSSMTLLVDAPGYDPLWFITSEPTQ

SEQ ID NO: 31 - protein, 51 aa, synthetic construct
IRKPNRQGLGYYSPSYNDPCSLQCPYLGSQSWTCPYTAPVSTPSWNFHSDV

SEQ ID NO: 32 - protein, 204 aa, synthetic construct
SRCTLTVGISSYHSSPCSPTQPVCTWNLDLNSLTTDQRLHPPCPNLITYSGFHKTYSLYLFPHWIKKPNRQGLGYYSPSYNDPCSLQCPYLGCQSWTCPYTGPVSSPSWKFHSDVNFTQEVSQVSLRLHFSKCGSSMTLLVDAPGYDPLWFITSEPTQPPPTSPPLVHDSDLEHVLTPSTSWTTKILKFIQLTLQSTNYSCMVC

SEQ ID NO: 33 - protein, 158 aa, synthetic construct
SRCTLTVGISSYHSSPCSPTQPVCTWNLDLNSLTTDQRLHPPCPNLITYSGFHKTYSLYLFPHWIKKPNRQGLGYYSPSYNDPCSLQCPYLGCQSWTCPYTGPVSSPSWKFHSDVNFTQEVSQVSLRLHFSKCGSSMTLLVDAPGYDPLWFITSEPTQ

SEQ ID NO: 34 - protein, 315 aa, synthetic construct
MGKSGLYFSLICFYTLFPSSFGNPSRCTLFIGASSYHSDPCGSNHPRCTWRLDLFSLTKDQSLSPPCPGLVTYSQYHKPYSLYVFPHWIAKPDRRGLGYYSASYSDPCAIQCPYLGCQSWTCPYTGPVSNPHWKYTSDLNFTQEVSSISLHLHFSKCGSSFSFLLDAPGYDPVWLLSSQATQIPPTPAPLIQDSDLQHILEPSIPWSSKILNLILLALKSTNYSCMVCVDRSSLSSWHVLYDPLKAPSSPDPQAQSILRPSLAIPASNITPPFPWTHCYRPPLQAISSENCNNSVILPPFSLSPIPDVSRPRKRR

SEQ ID NO: 35 - protein, 293 aa, synthetic construct
NPSRCTLFIGASSYHSDPCGSNHPRCTWRLDLFSLTKDQSLSPPCPGLVTYSQYHKPYSLYVFPHWIAKPDRRGLGYYSASYSDPCAIQCPYLGCQSWTCPYTGPVSNPHWKYTSDLNFTQEVSSISLHLHFSKCGSSFSFLLDAPGYDPVWLLSSQATQIPPTPAPLIQDSDLQHILEPSIPWSSKILNLILLALKSTNYSCMVCVDRSSLSSWHVLYDPLKAPSSPDPQAQSILRPSLAIPASNITPPFPWTHCYRPPLQAISSENCNNSVILPPFSLSPIPDVSRPRKRR

SEQ ID NO: 36 - protein, 180 aa, synthetic construct
MGKSGLYFSLICFYTLFPSSFGNPSRCTLFIGASSYHSDPCGSNHPRCTWRLDLFSLTKDQSLSPPCPGLVTYSQYHKPYSLYVFPHWIAKPDRRGLGYYSASYSDPCAIQCPYLGCQSWTCPYTGPVSNPHWKYTSDLNFTQEVSSISLHLHFSKCGSSFSFLLDAPGYDPVWLLSSQA

SEQ ID NO: 37 - protein, 158 aa, synthetic construct
NPSRCTLFIGASSYHSDPCGSNHPRCTWRLDLFSLTKDQSLSPPCPGLVTYSQYHKPYSLYVFPHWIAKPDRRGLGYYSASYSDPCAIQCPYLGCQSWTCPYTGPVSNPHWKYTSDLNFTQEVSSISLHLHFSKCGSSFSFLLDAPGYDPVWLLSSQA

SEQ ID NO: 38 - protein, 307 aa, synthetic construct
MGNVLFLTLLATLGIPVLQASRCTITVGISSYHSSPCSPAQPLCTWALDLVSITKDQLLYPPCQNLITYSNYHKTYSLYLFPHWVQKPLRRGLGYYSASYSDPCSLQCPYLGSQSWTCPYTGPVSSPTWRFSTDVNFTQEVSRVSLKLHFSKCGSSLTLLIDAPGYDPLWYLTSEPTQEPPTPPPLVSDSDLEHVLTPSASWASKMLTLIHLTLQSTNYSCMVCIDRASLSSWHVLYTPNISSNAPSKPIVRPSLALSAPRPQPFPWTHCYQPQVQAVTTAKCNNSIILPPFSLSPLPGAPLTRRRR

SEQ ID NO: 39 - protein, 287 aa, synthetic construct
SRCTITVGISSYHSSPCSPAQPLCTWALDLVSITKDQLLYPPCQNLITYSNYHKTYSLYLFPHWVQKPLRRGLGYYSASYSDPCSLQCPYLGSQSWTCPYTGPVSSPTWRFSTDVNFTQEVSRVSLKLHFSKCGSSLTLLIDAPGYDPLWYLTSEPTQEPPTPPPLVSDSDLEHVLTPSASWASKMLTLIHLTLQSTNYSCMVCIDRASLSSWHVLYTPNISSNAPSKPIVRPSLALSAPRPQPFPWTHCYQPQVQAVTTAKCNNSIILPPFSLSPLPGAPLTRRRR

SEQ ID NO: 40 - protein, 224 aa, synthetic construct
MGNVLFLTLLATLGIPVLQASRCTITVGISSYHSSPCSPAQPLCTWALDLVSITKDQLLYPPCQNLITYSNYHKTYSLYLFPHWVQKPLRRGLGYYSASYSDPCSLQCPYLGSQSWTCPYTGPVSSPTWRFSTDVNFTQEVSRVSLKLHFSKCGSSLTLLIDAPGYDPLWYLTSEPTQEPPTPPPLVSDSDLEHVLTPSASWASKMLTLIHLTLQSTNYSCMVC

SEQ ID NO: 41 - protein, 178 aa, synthetic construct
MGNVLFLTLLATLGIPVLQASRCTITVGISSYHSSPCSPAQPLCTWALDLVSITKDQLLYPPCQNLITYSNYHKTYSLYLFPHWVQKPLRRGLGYYSASYSDPCSLQCPYLGSQSWTCPYTGPVSSPTWRFSTDVNFTQEVSRVSLKLHFSKCGSSLTLLIDAPGYDPLWYLTSEPTQ

SEQ ID NO: 42 - protein, 204 aa, synthetic construct
SRCTITVGISSYHSSPCSPAQPLCTWALDLVSITKDQLLYPPCQNLITYSNYHKTYSLYLFPHWVQKPLRRGLGYYSASYSDPCSLQCPYLGSQSWTCPYTGPVSSPTWRFSTDVNFTQEVSRVSLKLHFSKCGSSLTLLIDAPGYDPLWYLTSEPTQEPPTPPPLVSDSDLEHVLTPSASWASKMLTLIHLTLQSTNYSCMVC

SEQ ID NO: 43 - protein, 158 aa, synthetic construct
SRCTITVGISSYHSSPCSPAQPLCTWALDLVSITKDQLLYPPCQNLITYSNYHKTYSLYLFPHWVQKPLRRGLGYYSASYSDPCSLQCPYLGSQSWTCPYTGPVSSPTWRFSTDVNFTQEVSRVSLKLHFSKCGSSLTLLIDAPGYDPLWYLTSEPTQ

SEQ ID NO: 44 - protein, 312 aa, synthetic construct
MGKFLATLILFFQFCPLILGDYSPSCCTLTIGVSSYLSKPCNPAQPVCSWTLDLLALSADQALQPPCPNLVSYSSYHATYSLYLFPHWIKKPNRNGGGYYSASYSDPCSLKCPYLGCQSWTCPYTGVVSSPYWKFQQDVNFTQEVSHLNINLHFSKCGFPFSLLIDAPGYDPIWFLNTEPSQLPPTAPPLLPHSNLDHILEPSIPWKSKLLTLVQLTLQSTNYTCIVCIDRASLSTWHVLYSPNVSVPSSSSTPLLYPSLALPAPHLTLPFNWTHCFDPQIQAIVSSPCHNSLILPPFSLSPVPTLGSRSRR

SEQ ID NO: 45 - protein, 292 aa, synthetic construct
DYSPSCCTLTIGVSSYLSKPCNPAQPVCSWTLDLLALSADQALQPPCPNLVSYSSYHATYSLYLFPHWIKKPNRNGGGYYSASYSDPCSLKCPYLGCQSWTCPYTGVVSSPYWKFQQDVNFTQEVSHLNINLHFSKCGFPFSLLIDAPGYDPIWFLNTEPSQLPPTAPPLLPHSNLDHILEPSIPWKSKLLTLVQLTLQSTNYTCIVCIDRASLSTWHVLYSPNVSVPSSSSTPLLYPSLALPAPHLTLPFNWTHCFDPQIQAIVSSPCHNSLILPPFSLSPVPTLGSRSRR

SEQ ID NO: 46 - protein, 179 aa, synthetic construct
MGKFLATLILFFQFCPLILGDYSPSCCILTIGVSSYHSKPCNPAQPVCSWTLDLLALSADQALQPPCPNLVSYSSYHATYSLYLFPHWIKKPNRNGGGYYSASYSDPCSLKCPYLGCQSWTCPYTGAVSSPYWKFQQDVNFTQEVSHLNINLHFSKCGFPFSLLIDAPGYDPIWFLNTE

SEQ ID NO: 47 - protein, 159 aa, synthetic construct
DYSPSCCILTIGVSSYHSKPCNPAQPVCSWTLDLLALSADQALQPPCPNLVSYSSYHATYSLYLFPHWIKKPNRNGGGYYSASYSDPCSLKCPYLGCQSWTCPYTGAVSSPYWKFQQDVNFTQEVSHLNINLHFSKCGFPFSLLIDAPGYDPIWFLNTE

SEQ ID NO: 48 - protein, 308 aa, synthetic construct
MGKIIAFLLFHLTCITITKQSRCTLTVGVSSYHSSPCSLAQPICTWDLDLHSLTTDQRLYPPCPNLVSYSNFHKSYSLYLFPHWVKKPNRQGLGYYSASYSDPCSLQCPYLGSQSWTCPYTGPISSPSWRFHRDVNFTQEVNHVTLRLHFSRCGSSMTLLIDAPGYDPLWFISSEPTQPPPTSPPLVRDSDLEHILTPSSSWATRMLTLIQLTLQSTNYSCMVCIDRTSLSSWHVLYTPNISASPGGDSLPILYPSLALPAPQPQPFSWSHCYQPHLQAVTTANCNNSIVLPPFSLTPVPSPGTRSRR

SEQ ID NO: 49 - protein, 288 aa, synthetic construct
SRCTLTVGVSSYHSSPCSLAQPICTWDLDLHSLTTDQRLYPPCPNLVSYSNFHKSYSLYLFPHWVKKPNRQGLGYYSASYSDPCSLQCPYLGSQSWTCPYTGPISSPSWRFHRDVNFTQEVNHVTLRLHFSRCGSSMTLLIDAPGYDPLWFISSEPTQPPPTSPPLVRDSDLEHILTPSSSWATRMLTLIQLTLQSTNYSCMVCIDRTSLSSWHVLYTPNISASPGGDSLPILYPSLALPAPQPQPFSWSHCYQPHLQAVTTANCNNSIVLPPFSLTPVPSPGTRSRR

SEQ ID NO: 50 - protein, 175 aa, synthetic construct
MGKIIAFLLFHLTCITITKQSRCTLTVGVSSYHSSPCSLAQPICTWDLDLHSLTTDQRLYPPCPNLVSYSNFHKSYSLYLFPHWVKKPNRQGLGYYSASYSDPCSLQCPYLGSQSWTCPYTGPISSPSWRFHRDVNFTQEVNHVTLRLHFSRCGSSMTLLIDAPGYDPLWFISSE

SEQ ID NO: 51 - protein, 155 aa, synthetic construct
SRCTLTVGVSSYHSSPCSLAQPICTWDLDLHSLTTDQRLYPPCPNLVSYSNFHKSYSLYLFPHWVKKPNRQGLGYYSASYSDPCSLQCPYLGSQSWTCPYTGPISSPSWRFHRDVNFTQEVNHVTLRLHFSRCGSSMTLLIDAPGYDPLWFISSE

SEQ ID NO: 52 - protein, 314 aa, synthetic construct
MGKFGLYCLVHLYILLPASSGNPSRCTLFIGASSYHSSPCGSSLPRCTWNLDLFSLTKDQSLSPPCPDLITYSQYHKPYSLYVFPHWITKPNRRGLGYYSASYSDPCAIQCPYLGCQSWTCPYTGPVSSPHWRYTYDLNFTQEVSSVSLHLHFSKCGSSFSFLLDAPGYDPVWFLSSQATQAPPTPAPLIRDSDLQYILEPPIPWSSKILNLILLTLKSTNYSCMVCVDRSSLSSWHVLYGPTQVPSPPDPQARSILRPALAIPASNITPPFPWTHCYRPPPQAISSENCNNSVVLPPFSLSPIPNVSRPRKRR

SEQ ID NO: 53 - protein, 293 aa, synthetic construct
NPSRCTLFIGASSYHSSPCGSSLPRCTWNLDLFSLTKDQSLSPPCPDLITYSQYHKPYSLYVFPHWITKPNRRGLGYYSASYSDPCAIQCPYLGCQSWTCPYTGPVSSPHWRYTYDLNFTQEVSSVSLHLHFSKCGSSFSFLLDAPGYDPVWFLSSQATQAPPTPAPLIRDSDLQYILEPPIPWSSKILNLILLTLKSTNYSCMVCVDRSSLSSWHVLYGPTQVPSPPDPQARSILRPALAIPASNITPPFPWTHCYRPPPQAISSENCNNSVVLPPFSLSPIPNVSRPRKRR

SEQ ID NO: 54 - protein, 181 aa, synthetic construct
MGKSGFYFCFIYTLFPASFGNPSRCTLFIGASSYHSDPCGSNHPQCTWRLDLFSLTRDQSLSPPCPDLVTYSQYHKPYSLYVFPHWMAKPNRQGLGYYSASYSDPCAIQCPYLGCQSWTCPYTGPVSSPHWKYSSDLNFTQEVSSISLHLHFSKCGSSFSFLLDAPGYDPVWFLSSQATQV

SEQ ID NO: 55 - protein, 161 aa, synthetic construct
NPSRCTLFIGASSYHSDPCGSNHPQCTWRLDLFSLTRDQSLSPPCPDLVTYSQYHKPYSLYVFPHWMAKPNRQGLGYYSASYSDPCAIQCPYLGCQSWTCPYTGPVSSPHWKYSSDLNFTQEVSSISLHLHFSKCGSSFSFLLDAPGYDPVWFLSSQATQV

SEQ ID NO: 56 - protein, 312 aa, synthetic construct
MGKSLFFFCIIVQACLPTLCDRGPSCCTLTVGVSSYHSKPCNPTQPICSWTLDLLTLTTDQALQPPCPNLIGYSNYHATYPLYLFPHWVKKPNRGGGGYYSASYSDPCSLKCPYLGCQSWTCPYTGAVSGPYWKYQTDVNFTQDVSRLTVHLHFSKCGFPFSLLIDAPGYDPIWLINSEPSQLPPTAPPLLPHSNLDHILEPSIPWKSKLLTLVQLTLQSTNYTCIVCLDRASLSTWHVLYSPNMSVPSSPSVPLIYPSLALPAPHLALPFNWTHCFDPKLQAITSAHCYNALILPPFSLSPVPALSHRTRR

SEQ ID NO: 57 - protein, 293 aa, synthetic construct
CDRGPSCCTLTVGVSSYHSKPCNPTQPICSWTLDLLTLTTDQALQPPCPNLIGYSNYHATYPLYLFPHWVKKPNRGGGGYYSASYSDPCSLKCPYLGCQSWTCPYTGAVSGPYWKYQTDVNFTQDVSRLTVHLHFSKCGFPFSLLIDAPGYDPIWLINSEPSQLPPTAPPLLPHSNLDHILEPSIPWKSKLLTLVQLTLQSTNYTCIVCLDRASLSTWHVLYSPNMSVPSSPSVPLIYPSLALPAPHLALPFNWTHCFDPKLQAITSAHCYNALILPPFSLSPVPALSHRTRR

SEQ ID NO: 58 - protein, 178 aa, synthetic construct; identical to SEQ ID NO: 30

SEQ ID NO: 59 - protein, 228 aa, synthetic construct
APSTCSKPTCPPPELLGGPSVFIFPPKPKDTLMISRTPEVTCVVVDVSQDDPEVQFTWYINNEQVRTARPPLREQQFDCTIRVVSTLPIAHQDWLRGKEFKCKVHNKALPAPIEKTISKARGQPLEPKVYTMGPPREELSSRSVSLTCMINGFYPSDISVEWEKNGKAEDNYKTTPAVLDSDGSYFLYSKLSVPTSEWQRGDVFTCSVMHEALHNHYTQKSISRSPGK

SEQ ID NO: 60 - protein, 229 aa, synthetic construct
VDVPRDCGCKPCICTVPEVSSVFIFPPKPKDVLTITLTPKVTCVVVDISKDDPEVQFSWFVDDVEVHTAQTQPREEQFNSTFRSVSELPIMHQDWLNGKEFKCRVNSAAFPAPIEKTISKTKGRPKAPQVYTIPPPKEQMAKDKVSLTCMITDFFPEDITVEWQWNGQPAENYKNTQPIMDTDGSYFVYSKLNVQKSNWEAGNTFTCSVLHEGLHNHHTEKSLSHSPGK

SEQ ID NO: 61 - protein, 352 aa, synthetic construct
MALPYHIFLFTVLLPSFTLTAPPPCRCMTSSSPYQEFLWRMQRPGNIDAPSYRSLSKGTPTFTAHTHMPRNCYHSATLCMHANTHYWTGKMINPSCPGGLGVTVCWTYFTQTGMSDGGGVQGSVDVPRDCGCKPCICTVPEVSSVFIFPPKPKDVLTITLTPKVTCVVVDISKDDPEVQFSWFVDDVEVHTAQTQPREEQFNSTFRSVSELPIMHQDWLNGKEFKCRVNSAAFPAPIEKTISKTKGRPKAPQVYTIPPPKEQMAKDKVSLTCMITDFFPEDITVEWQWNGQPAENYKNTQPIMDTDGSYFVYSKLNVQKSNWEAGNTFTCSVLHEGLHNHHTEKSLSHSPGK

SEQ ID NO: 62 - protein, 453 aa, synthetic construct
MKLPTGMVILCSLIIVRAGFDDPRKAIALVQKQHGKPCECSGGQVSEAPPNSIQQVTCPGKTAYLMTNQKWKCRVTPKISPSGGELQNCPCNTFQDSMHSSCYTEYRQCRRINKTYYTATLLKIRSGSLNEVQILQNPNQLLQSPCRGSINQPVCWSATAPIHISDGGGPLDTKRVWTVQKRLEQIHKAMTPELQYHPLALPKVRDDLSLDARTFDILNTTFGSVDVPRDCGCKPCICTVPEVSSVFIFPPKPKDVLTITLTPKVTCVVVDISKDDPEVQFSWFVDDVEVHTAQTQPREEQFNSTFRSVSELPIMHQDWLNGKEFKCRVNSAAFPAPIEKTISKTKGRPKAPQVYTIPPPKEQMAKDKVSLTCMITDFFPEDITVEWQWNGQPAENYKNTQPIMDTDGSYFVYSKLNVQKSNWEAGNTFTCSVLHEGLHNHHTEKSLSHSPGK

SEQ ID NO: 63 - protein, 454 aa, synthetic construct
MKLPAGMVILCSLIIVRAGFDDPRKAIALVQKQHGKPCECSGGQVSEAPPNSIQQVTCPGKTAYLMTNQKWKCRVTPKNLTPSGGELQNCPCNTFQDSMHSSCYTEYRQCRANNKTYYTATLLKIRSGSLNEVQILQNPNQLLQSPCRGSINQPVCWSATAPIHISDGGGPLDTKRVWTVQKRLEQIHKAMHPELQYHPLALPKVRDDLSLDARTFDILNTTFGSVDVPRDCGCKPCICTVPEVSSVFIFPPKPKDVLTITLTPKVTCVVVDISKDDPEVQFSWFVDDVEVHTAQTQPREEQFNSTFRSVSELPIMHQDWLNGKEFKCRVNSAAFPAPIEKTISKTKGRPKAPQVYTIPPPKEQMAKDKVSLTCMITDFFPEDITVEWQWNGQPAENYKNTQPIMDTDGSYFVYSKLNVQKSNWEAGNTFTCSVLHEGLHNHHTEKSLSHSPGK

SEQ ID NO: 64 - protein, 408 aa, synthetic construct
MGNVFFLLLFSLTHFPLAQQSRCTLTVGISSYHSSPCSPTQPVCTWNLDLNSLTTDQRLHPPCPNLITYSGFHKTYSLYLFPHWIKKPNRQGLGYYSPSYNDPCSLQCPYLGCQSWTCPYTGPVSSPSWKFHSDVNFTQEVSQVSLRLHFSKCGSSMTLLVDAPGYDPLWFITSEPTQGSAPSTCSKPTCPPPELLGGPSVFIFPPKPKDTLMISRTPEVTCVVVDVSQDDPEVQFTWYINNEQVRTARPPLREQQFDCTIRVVSTLPIAHQDWLRGKEFKCKVHNKALPAPIEKTISKARGQPLEPKVYTMGPPREELSSRSVSLTCMINGFYPSDISVEWEKNGKAEDNYKTTPAVLDSDGSYFLYSKLSVPTSEWQRGDVFTCSVMHEALHNHYTQKSISRSPGK

SEQ ID NO: 65 - protein, 388 aa, synthetic construct
SRCTLTVGISSYHSSPCSPTQPVCTWNLDLNSLTTDQRLHPPCPNLITYSGFHKTYSLYLFPHWIKKPNRQGLGYYSPSYNDPCSLQCPYLGCQSWTCPYTGPVSSPSWKFHSDVNFTQEVSQVSLRLHFSKCGSSMTLLVDAPGYDPLWFITSEPTQGSAPSTCSKPTCPPPELLGGPSVFIFPPKPKDTLMISRTPEVTCVVVDVSQDDPEVQFTWYINNEQVRTARPPLREQQFDCTIRVVSTLPIAHQDWLRGKEFKCKVHNKALPAPIEKTISKARGQPLEPKVYTMGPPREELSSRSVSLTCMINGFYPSDISVEWEKNGKAEDNYKTTPAVLDSDGSYFLYSKLSVPTSEWQRGDVFTCSVMHEALHNHYTQKSISRSPGK

SEQ ID NO: 66 - protein, 409 aa, synthetic construct
MGNVFFLLLFSLTHFPLAQQSRCTLTVGISSYHSSPCSPTQPVCTWNLDLNSLTTDQRLHPPCPNLITYSGFHKTYSLYLFPHWIKKPNRQGLGYYSPSYNDPCSLQCPYLGCQSWTCPYTGPVSSPSWKFHSDVNFTQEVSQVSLRLHFSKCGSSMTLLVDAPGYDPLWFITSEPTQGSVDVPRDCGCKPCICTVPEVSSVFIFPPKPKDVLTITLTPKVTCVVVDISKDDPEVQFSWFVDDVEVHTAQTQPREEQFNSTFRSVSELPIMHQDWLNGKEFKCRVNSAAFPAPIEKTISKTKGRPKAPQVYTIPPPKEQMAKDKVSLTCMITDFFPEDITVEWQWNGQPAENYKNTQPIMDTDGSYFVYSKLNVQKSNWEAGNTFTCSVLHEGLHNHHTEKSLSHSPGK

SEQ ID NO: 67 - protein, 389 aa, synthetic construct
SRCTLTVGISSYHSSPCSPTQPVCTWNLDLNSLTTDQRLHPPCPNLITYSGFHKTYSLYLFPHWIKKPNRQGLGYYSPSYNDPCSLQCPYLGCQSWTCPYTGPVSSPSWKFHSDVNFTQEVSQVSLRLHFSKCGSSMTLLVDAPGYDPLWFITSEPTQGSVDVPRDCGCKPCICTVPEVSSVFIFPPKPKDVLTITLTPKVTCVVVDISKDDPEVQFSWFVDDVEVHTAQTQPREEQFNSTFRSVSELPIMHQDWLNGKEFKCRVNSAAFPAPIEKTISKTKGRPKAPQVYTIPPPKEQMAKDKVSLTCMITDFFPEDITVEWQWNGQPAENYKNTQPIMDTDGSYFVYSKLNVQKSNWEAGNTFTCSVLHEGLHNHHTEKSLSHSPGK

SEQ ID NO: 68 - protein, 418 aa, synthetic construct
MGNVFFLLLFSLTHFPLAQQSRCTLTVGISSYHSSPCSPTQPVCTWNLDLNSLTTDQRLHPPCPNLITYSGFHKTYSLYLFPHWIKKPNRQGLGYYSPSYNDPCSLQCPYLGCQSWTCPYTGPVSSPSWKFHSDVNFTQEVSQVSLRLHFSKCGSSMTLLVDAPGYDPLWFITSEPTQGSVSKGEELFTGVVPILVELDGDVNGHKFSVSGEGEGDATYGKLTLKFICTTGKLPVPWPTLVTTLTYGVQCFSRYPDHMKQHDFFKSAMPEGYVQERTIFFKDDGNYKTRAEVKFEGDTLVNRIELKGIDFKEDGNILGHKLEYNYNSHNVYIMADKQKNGIKVNFKIRHNIEDGSVQLADHYQQNTPIGDGPVLLPDNHYLSTQSALSKDPNEKRDHMVLLEFVTAAGITLGMDELYK

SEQ ID NO: 69 - protein, 398 aa, synthetic construct
SRCTLTVGISSYHSSPCSPTQPVCTWNLDLNSLTTDQRLHPPCPNLITYSGFHKTYSLYLFPHWIKKPNRQGLGYYSPSYNDPCSLQCPYLGCQSWTCPYTGPVSSPSWKFHSDVNFTQEVSQVSLRLHFSKCGSSMTLLVDAPGYDPLWFITSEPTQGSVSKGEELFTGVVPILVELDGDVNGHKFSVSGEGEGDATYGKLTLKFICTTGKLPVPWPTLVTTLTYGVQCFSRYPDHMKQHDFFKSAMPEGYVQERTIFFKDDGNYKTRAEVKFEGDTLVNRIELKGIDFKEDGNILGHKLEYNYNSHNVYIMADKQKNGIKVNFKIRHNIEDGSVQLADHYQQNTPIGDGPVLLPDNHYLSTQSALSKDPNEKRDHMVLLEFVTAAGITLGMDELYK

SEQ ID NO: 70 - protein, 541 aa, Homo sapiens
MVADPPRDSKGLAAAEPTANGGLALASIEDQGAAAGGYCGSRDQVRRCLRANLLVLLTVVAVVAGVALGLGVSGAGGALALGPERLSAFVFPGELLLRLLRMIILPLVVCSLIGGAASLDPGALGRLGAWALLFFLVTTLLASALGVGLALALQPGAASAAINASVGAAGSAENAPSKEVLDSFLDLARNIFPSNLVSAAFRSYSTTYEERNITGTRVKVPVGQEVEGMNILGLVVFAIVFGVALRKLGPEGELLIRFFNSFNEATMVLVSWIMWYAPVGIMFLVAGKIVEMEDVGLLFARLGKYILCCLLGHAIHGLLVLPLIYFLFTRKNPYRFLWGIVTPLATAFGTSSSSATLPLMMKCVEENNGVAKHISRFILPIGATVNMDGAALFQCVAAVFIAQLSQQSLDFVKIITILVTATASSVGAAGIPAGGVLTLAIILEAVNLPVDHISLILAVDWLVDRSCTVLNVEGDALGAGLLQNYVDRTESRSTEPELIQVKSELPLDPLPVPTEEGNPLLKHYRGPAGDATVASEKESVM

SEQ ID NO: 71 - protein, 492 aa, Homo sapiens
MEPSSKKLTGRLMLAVGGAVLGSLQFGYNTGVINAPQKVIEEFYNQTWVHRYGESILPTTLTTLWSLSVAIFSVGGMIGSFSVGLFVNRFGRRNSMLMMNLLAFVSAVLMGFSKLGKSFEMLILGRFIIGVYCGLTTGFVPMYVGEVSPTALRGALGTLHQLGIVVGILIAQVFGLDSIMGNKDLWPLLLSIIFIPALLQCIVLPFCPESPRFLLINRNEENRAKSVLKKLRGTADVTHDLQEMKEESRQMMREKKVTILELFRSPAYRQPILIAVVLQLSQQLSGINAVFYYSTSIFEKAGVQQPVYATIGSGIVNTAFTVVSLFVVERAGRRTLHLIGLAGMAGCAILMTIALALLEQLPWMSYLSIVAIFGFVAFFEVGPGPIPWFIVAELFSQGPRPAAIAVAGFSNWTSNFIVGMCFQYVEQLCGPYVFIIFTVLLVLFFIFTYFKVPETKGRTFDEIASGFRQGGASQSDKTPEELFHPLGADSQV